European Patent Application EP 4 682 255 A1, published January 21, 2026. Title: composition and use thereof. Applicant: TOAGOSEI CO., LTD. The sequence listing filed with the application follows.

SEQUENCE LISTING (13 sequences)

SEQ ID NO: 1 - RNA, 19 nt, synthetic construct
  source 1..19: mol_type = other RNA
gatatttgctgtctttata

SEQ ID NO: 2 - RNA, 19 nt, synthetic construct
  source 1..19: mol_type = other RNA
catttgctgaacgcattta

SEQ ID NO: 3 - RNA, 19 nt, synthetic construct
  source 1..19: mol_type = other RNA
cgtctgggcggtgctacaa

SEQ ID NO: 4 - protein, 18 aa, synthetic construct
MRIFAVFIFMTYWHLLNA

SEQ ID NO: 5 - DNA, 54 bp, synthetic construct
  source 1..54: mol_type = other DNA
atgaggatatttgctgtctttatattcatgacctactggcatttgctgaacgca

SEQ ID NO: 6 - protein, 23 aa, synthetic construct
MQIPQAPWPVVWAVLQLGWRPGW

SEQ ID NO: 7 - DNA, 69 bp, synthetic construct
  source 1..69: mol_type = other DNA
atgcagatcccacaggcgccctggccagtcgtctgggcggtgctacaactgggctggcggccaggatgg

SEQ ID NO: 8 - DNA, 21 bp, synthetic construct
  source 1..21: mol_type = other DNA
  misc_feature 1..19: note = RNA
  misc_feature 20..21: note = DNA
  modified_base 3: mod_base = OTHER; note = uracil
  modified_base 5..7: mod_base = OTHER; note = uracil
  modified_base 10: mod_base = OTHER; note = uracil
  modified_base 12: mod_base = OTHER; note = uracil
  modified_base 14..16: mod_base = OTHER; note = uracil
  modified_base 18: mod_base = OTHER; note = uracil
gatatttgctgtctttatatt

SEQ ID NO: 9 - DNA, 21 bp, synthetic construct
  misc_feature 1..19: note = RNA
  misc_feature 20..21: note = DNA
  source 1..21: mol_type = other DNA
  modified_base 1: mod_base = OTHER; note = uracil
  modified_base 3: mod_base = OTHER; note = uracil
  modified_base 16: mod_base = OTHER; note = uracil
  modified_base 18: mod_base = OTHER; note = uracil
tataaagacagcaaatatctt

SEQ ID NO: 10 - DNA, 21 bp, synthetic construct
  misc_feature 1..19: note = RNA
  misc_feature 20..21: note = DNA
  source 1..21: mol_type = other DNA
  modified_base 3..5: mod_base = OTHER; note = uracil
  modified_base 8: mod_base = OTHER; note = uracil
  modified_base 16..18: mod_base = OTHER; note = uracil
catttgctgaacgcatttatt

SEQ ID NO: 11 - DNA, 21 bp, synthetic construct
  misc_feature 1..19: note = RNA
  misc_feature 20..21: note = DNA
  source 1..21: mol_type = other DNA
  modified_base 1: mod_base = OTHER; note = uracil
  modified_base 5: mod_base = OTHER; note = uracil
  modified_base 9..10: mod_base = OTHER; note = uracil
  modified_base 18: mod_base = OTHER; note = uracil
taaatgcgttcagcaaatgtt

SEQ ID NO: 12 - DNA, 21 bp, synthetic construct
  misc_feature 1..19: note = RNA
  misc_feature 20..21: note = DNA
  source 1..21: mol_type = other DNA
  modified_base 3: mod_base = OTHER; note = uracil
  modified_base 5: mod_base = OTHER; note = uracil
  modified_base 12: mod_base = OTHER; note = uracil
  modified_base 15: mod_base = OTHER; note = uracil
cgtctgggcggtgctacaatt

SEQ ID NO: 13 - DNA, 21 bp, synthetic construct
  misc_feature 1..19: note = RNA
  misc_feature 20..21: note = DNA
  source 1..21: mol_type = other DNA
  modified_base 1..2: mod_base = OTHER; note = uracil
  modified_base 4: mod_base = OTHER; note = uracil
ttgtagcaccgcccagacgtt